European Patent Specification EP 3 076 987 B1, published July 12, 2023. Title: METHOD OF TREATING OR PREVENTING EPILEPSY OR SEIZURES USING ONE OR MORE NEURAL REGENERATION PEPTIDES. Applicant: Curonz Holdings Company Limited. The sequence listing filed with the application follows.

SEQUENCE LISTING (2 sequences)

SEQ ID NO: 1 - protein, 11 aa, Artificial sequence
  Peptide
  MOD_RES (9)..(9): Aib
GRRAAPGRXGG

SEQ ID NO: 2 - protein, 11 aa, Artificial sequence
  Peptide
  MOD_RES (9)..(9): Aib
  MOD_RES (11)..(11): AMIDATION
GRRAAPGRXGG